European Patent Application EP 4 414 443 A1, published August 14, 2024. Title: CLEANING COMPOSITION COMPRISING POLYESTERASE. Applicant: Henkel AG & Co. KGaA. The sequence listing filed with the application follows.

SEQUENCE LISTING (1 sequence)

SEQ ID NO: 1 - protein, 258 aa, Pseudomonas mendocina
APLPDTPGAPFPAVANFDRSGPYTVSSQSEGPSCRIYRPRDLGQGGVRHPVILWGNGTGAGPSTYAGLLSHWASHGFVVAAAETSNAGTGREMLACLDYLVRENDTPYGTYSGKLNTGRVGTSGHSQGGGGSIMAGQDTRVRTTAPIQPYTLGLGHDSASQRRQQGPMFLMSGGGDTIAFPYLNAQPVYRRANVPVFWGERRYVSHFEPVGSGGAYRGPSTAWFRFQLMDDQDARATFYGAQCSLCTSLLWSVERRGL